European Patent Application EP 4 748 451 A2, published May 27, 2026. Title: ANTISENSE OLIGONUCLEOTIDES AND USES THEREOF. Applicant: Fundació Centre de Regulació Genòmica. The sequence listing filed with the application follows.

SEQUENCE LISTING (357 sequences)

SEQ ID NO: 1 - DNA, 147 bp, Mus musculus
  misc_feature 1..147: note = Description of sequence: NM_001136075.2 - Numb mRNA transcript variant 1 1115..1261
  source 1..147: mol_type = genomic DNA
ctaatggcactgactcagcctcccatgtgcttactgctaagccagccaatactgctctagcacacgtagcaatgcctgtccgtgaaaccaacccctgggcccatgtccctgatgctgctaacaaggaaattgcagccatacatccgg

SEQ ID NO: 2 - DNA, 144 bp, Homo sapiens
  misc_feature 1..144: note = Description: NM_001005743 Numb mRNA transcript variant 1-1417..1560
  source 1..144: mol_type = genomic DNA
ctaatggcactgactcagccttccatgtgcttgctaagccagcccatactgctctagcacccgtagcaatgcctgtgcgtgaaaccaacccttgggcccatgcccctgatgctgctaacaaggaaattgcagccacatgttcgg

SEQ ID NO: 3 - RNA, 21 nt, Homo sapiens
  misc_feature 1..21: note = Description of sequence: Region 2 of Homo sapiens Numb exon 9 (targeted by AON2 - SEQ ID NO: 13)
  source 1..21: mol_type = genomic RNA
ccttccatgtgcttgctaagc

SEQ ID NO: 4 - RNA, 21 nt, Homo sapiens
  misc_feature 1..21: note = Description of sequence: Region 3 of Homo sapiens Numb exon 9 (targeted by AON3 - SEQ ID NO: 14)
  source 1..21: mol_type = genomic RNA
cagcccatactgctctagcac

SEQ ID NO: 5 - RNA, 21 nt, Homo sapiens
  misc_feature 1..21: note = Description of sequence: Region 4 of Homo sapiens Numb exon 9 (targeted by AON4 - SEQ ID NO: 15)
  source 1..21: mol_type = genomic RNA
ccgtagcaatgcctgtgcgtg

SEQ ID NO: 6 - RNA, 21 nt, Homo sapiens
  misc_feature 1..21: note = Description of sequence: Region 5 of Homo sapiens Numb exon 9 (targeted by AON5 - SEQ ID NO: 16)
  source 1..21: mol_type = genomic RNA
aaaccaacccttgggcccatg

SEQ ID NO: 7 - RNA, 21 nt, Homo sapiens
  misc_feature 1..21: note = Description of sequence: Region 6 of Homo sapiens Numb exon 9 (targeted by AON6 - SEQ ID NO: 17)
  source 1..21: mol_type = genomic RNA
cccctgatgctgctaacaagg

SEQ ID NO: 8 - RNA, 21 nt, Homo sapiens
  misc_feature 1..21: note = Description of sequence: Region 7 of Homo sapiens Numb exon 9 (targeted by AON7 - SEQ ID NO: 18)
  source 1..21: mol_type = genomic RNA
aaattgcagccacatgttcgg

SEQ ID NO: 9 - RNA, 39 nt, Homo sapiens
  misc_feature 1..39: note = Description of sequence: Region 1+2 of Homo sapiens Numb exon 9 (targeted by AON1 - SEQ ID NO: 12 ; AON2 - SEQ ID NO: 13; and AON1-2 - SEQ ID NO: 19)
  source 1..39: mol_type = genomic RNA
ctaatggcactgactcagccttccatgtgcttgctaagc

SEQ ID NO: 10 - RNA, 42 nt, Homo sapiens
  misc_feature 1..42: note = Description of sequence: Region 4+5 of Homo sapiens Numb exon 9 (targeted by AON4 - SEQ ID NO: 15; AON5 - SEQ ID NO:16; and AON4-5 - SEQ ID NO: 22)
  source 1..42: mol_type = genomic RNA
ccgtagcaatgcctgtgcgtgaaaccaacccttgggcccatg

SEQ ID NO: 11 - RNA, 42 nt, Homo sapiens
  misc_feature 1..42: note = Description of sequence: Region 6+7 of Homo sapiens Numb exon 9 (targeted by AON6 - SEQ ID NO: 17; AON7 - SEQ ID NO: 18 and AON6-7 - SEQ ID NO: 24)
  source 1..42: mol_type = genomic RNA
cccctgatgctgctaacaaggaaattgcagccacatgttcgg

SEQ ID NO: 12 - RNA, 21 nt, synthetic construct
  misc_feature 1..21: note = Description of sequence: Antisense oligonucleotide targeting region 1 of Homo sapiens Numb exon 9 (AON1)
  source 1..21: mol_type = other RNA
aggctgagtcagtgccattag

SEQ ID NO: 13 - RNA, 21 nt, synthetic construct
  misc_feature 1..21: note = Description of sequence: Antisense oligonucleotide targeting region 2 of Homo sapiens Numb exon 9 (AON2)
  source 1..21: mol_type = other RNA
gcttagcaagcacatggaagg

SEQ ID NO: 14 - RNA, 21 nt, synthetic construct
  misc_feature 1..21: note = Description of sequence: Antisense oligonucleotide targeting region 3 of Homo sapiens Numb exon 9 (AON3)
  source 1..21: mol_type = other RNA
gtgctagagcagtatgggctg

SEQ ID NO: 15 - RNA, 21 nt, synthetic construct
  misc_feature 1..21: note = Description of sequence: Antisense oligonucleotide targeting region 4 of Homo sapiens Numb exon 9 (AON4)
  source 1..21: mol_type = other RNA
cacgcacaggcattgctacgg

SEQ ID NO: 16 - RNA, 21 nt, synthetic construct
  misc_feature 1..21: note = Description of sequence: Antisense oligonucleotide targeting region 5 of Homo sapiens Numb exon 9 (AON5)
  source 1..21: mol_type = other RNA
catgggcccaagggttggttt

SEQ ID NO: 17 - RNA, 21 nt, synthetic construct
  misc_feature 1..21: note = Description of sequence: Antisense oligonucleotide targeting region 6 of Homo sapiens Numb exon 9 (AON6)
  source 1..21: mol_type = other RNA
ccttgttagcagcatcagggg

SEQ ID NO: 18 - RNA, 21 nt, synthetic construct
  misc_feature 1..21: note = Description of sequence: Antisense oligonucleotide targeting region 7 of Homo sapiens Numb exon 9 (AON7)
  source 1..21: mol_type = other RNA
ccgaacatgtggctgcaattt

SEQ ID NO: 19 - RNA, 21 nt, synthetic construct
  misc_feature 1..21: note = Description of sequence: Antisense oligonucleotide targeting region 1-2 of Homo sapiens Numb exon 9 (AON1-2)
  source 1..21: mol_type = other RNA
cacatggaaggctgagtcagt

SEQ ID NO: 20 - RNA, 21 nt, synthetic construct
  misc_feature 1..21: note = Description of sequence: Antisense oligonucleotide targeting region 2-3 of Homo sapiens Numb exon 9 (AON2-3)
  source 1..21: mol_type = other RNA
agtatgggctggcttagcaag

SEQ ID NO: 21 - RNA, 21 nt, synthetic construct
  misc_feature 1..21: note = Description of sequence: Antisense oligonucleotide targeting region 3-4 of Homo sapiens Numb exon 9 (AON3-4)
  source 1..21: mol_type = other RNA
cattgctacgggtgctagagc

SEQ ID NO: 22 - RNA, 21 nt, synthetic construct
  misc_feature 1..21: note = Description of sequence: Antisense oligonucleotide targeting region 4-5 of Homo sapiens Numb exon 9 (AON4-5)
  source 1..21: mol_type = other RNA
agggttggtttcacgcacagg

SEQ ID NO: 23 - RNA, 21 nt, synthetic construct
  misc_feature 1..21: note = Description of sequence: Antisense oligonucleotide targeting region 5-6 of Homo sapiens Numb exon 9 (AON5-6)
  source 1..21: mol_type = other RNA
agcatcaggggcatgggccca

SEQ ID NO: 24 - RNA, 21 nt, synthetic construct
  misc_feature 1..21: note = Description of sequence: Antisense oligonucleotide targeting region 6-7 of Homo sapiens Numb exon 9 (AON6-7)
  source 1..21: mol_type = other RNA
ggctgcaatttccttgttagc

SEQ ID NO: 25 - RNA, 21 nt, synthetic construct
  misc_feature 1..21: note = Description of sequence: Antisense oligonucleotide targeting the 5' splice site of Numb exon 9
  source 1..21: mol_type = other RNA
atctgtggccaccttacccga

SEQ ID NO: 26 - RNA, 21 nt, synthetic construct
  misc_feature 1..21: note = Description of sequence: Antisense oligonucleotide targeting the 3' splice site of Homo sapiens Numb exon 9
  source 1..21: mol_type = other RNA
ttagctacaacgggagcagac

SEQ ID NO: 27 - RNA, 21 nt, Homo sapiens
  misc_feature 1..21: note = Description of sequence: Homo sapiens Numb exon 9 sequence targeted by antisense oligonucleotide of SEQ. ID NO: 25
  source 1..21: mol_type = genomic RNA
tcgggtaaggtggccacagat

SEQ ID NO: 28 - RNA, 21 nt, Homo sapiens
  misc_feature 1..21: note = Description of sequence: Homo sapiens Numb exon 9 sequence targeted by antisense oligonucleotide of SEQ. ID NO: 26
  misc_feature 2: note = r-Thymine
  misc_feature 4: note = r-Thymine
  misc_feature 6: note = r-Thymine
  misc_feature 12: note = r-Thymine
  misc_feature 13: note = r-Thymine
  misc_feature 15: note = r-Thymine
  misc_feature 19: note = r-Thymine
  source 1..21: mol_type = genomic RNA
gtctgctcccgttgtagctaa

SEQ ID NO: 29 - RNA, 23 nt, synthetic construct
  misc_feature 1..23: note = Description of sequence: Antisense oligonucleotide targeting the branching point of Homo sapiens Numb exon 9
  source 1..23: mol_type = other RNA
caacatcaatggagttaattcat

SEQ ID NO: 30 - RNA, 21 nt, Homo sapiens
  misc_feature 1..21: note = Description of sequence: Region of Homo sapiens Numb exon 9 targeted by SEQ.ID NO: 19 (AON1-2)
  source 1..21: mol_type = genomic RNA
actgactcagccttccatgtg

SEQ ID NO: 31 - RNA, 21 nt, Homo sapiens
  misc_feature 1..21: note = Description of sequence: Region of Homo sapiens Numb exon 9 targeted by SEQ.ID NO: 22 (AON4-5)
  source 1..21: mol_type = genomic RNA
cctgtgcgtgaaaccaaccct

SEQ ID NO: 32 - RNA, 21 nt, Homo sapiens
  misc_feature 1..21: note = Description of sequence: Region of Homo sapiens Numb exon 9 targeted by SEQ.ID NO: 24 (AON6-7)
  source 1..21: mol_type = genomic RNA
gctaacaaggaaattgcagcc

SEQ ID NO: 33 - RNA, 21 nt, Homo sapiens
  misc_feature 1..21: note = Description of sequence: Region of Homo sapiens Numb exon 9 targeted by SEQ.ID NO: 20 (AON2-3)
  source 1..21: mol_type = genomic RNA
cttgctaagccagcccatact

SEQ ID NO: 34 - RNA, 21 nt, Homo sapiens
  misc_feature 1..21: note = Description of sequence: Region of Homo sapiens Numb exon 9 targeted by SEQ.ID NO: 21 (AON3-4)
  source 1..21: mol_type = genomic RNA
gctctagcacccgtagcaatg

SEQ ID NO: 35 - RNA, 21 nt, Homo sapiens
  misc_feature 1..21: note = Description of sequence: Region of Homo sapiens Numb exon 9 targeted by SEQ.ID NO: 23 (AON5-6)
  source 1..21: mol_type = genomic RNA
tgggcccatgcccctgatgct

SEQ ID NO: 36-40 - skipped (5 entries)

SEQ ID NO: 41 - RNA, 14 nt, synthetic construct
  misc_feature 1..14: note = Description for SEQ ID NO:41: Antisense oligonucleotide targeting region 1 of Homo sapiens Numb exon 9
  source 1..14: mol_type = other RNA
aggctgagtcagtg

SEQ ID NO: 42 - RNA, 14 nt, synthetic construct
  misc_feature 1..14: note = Description for SEQ ID NO:42: Antisense oligonucleotide targeting region 1 of Homo sapiens Numb exon 9
  source 1..14: mol_type = other RNA
gtcagtgccattag

SEQ ID NO: 43 - RNA, 21 nt, synthetic construct
  misc_feature 1..21: note = Description for SEQ ID NO:43: Antisense oligonucleotide targeting region 1 of Homo sapiens Numb exon 9
  modified_base 4: mod_base = cm
  modified_base 10: mod_base = cm
  modified_base 15: mod_base = cm
  modified_base 16: mod_base = cm
  source 1..21: mol_type = other RNA
aggctgagtcagtgccattag

SEQ ID NO: 44 - RNA, 21 nt, Homo sapiens
  misc_feature 1..21: note = Description for SEQ ID NO:44: Region 1 of Homo sapiens Numb exon 9 (targeted by AON1 - SEQ ID NO:12)
  source 1..21: mol_type = genomic RNA
ctaatggcactgactcagcct

SEQ ID NO: 45-77 - skipped (33 entries)

SEQ ID NO: 78 - RNA, 13 nt, Homo sapiens
  misc_feature 1..13: note = Description for SEQ ID NO:78: target regions in region 1+2 of homo sapiens numb exon 9
  source 1..13: mol_type = genomic RNA
ctaatggcactga

SEQ ID NO: 79 - RNA, 13 nt, Homo sapiens
  misc_feature 1..13: note = Description for SEQ ID NO:79: target regions in region 1+2 of homo sapiens numb exon 9
  source 1..13: mol_type = genomic RNA
taatggcactgac

SEQ ID NO: 80 - RNA, 13 nt, Homo sapiens
  misc_feature 1..13: note = Description for SEQ ID NO:80: target regions in region 1+2 of homo sapiens numb exon 9
  source 1..13: mol_type = genomic RNA
aatggcactgact

SEQ ID NO: 81 - RNA, 13 nt, Homo sapiens
  misc_feature 1..13: note = Description for SEQ ID NO:81: target regions in region 1+2 of homo sapiens numb exon 9
  source 1..13: mol_type = genomic RNA
atggcactgactc

SEQ ID NO: 82 - RNA, 13 nt, Homo sapiens
  misc_feature 1..13: note = Description for SEQ ID NO:82: target regions in region 1+2 of homo sapiens numb exon 9
  source 1..13: mol_type = genomic RNA
tggcactgactca

SEQ ID NO: 83 - RNA, 13 nt, Homo sapiens
  misc_feature 1..13: note = Description for SEQ ID NO:83: target regions in region 1+2 of homo sapiens numb exon 9
  source 1..13: mol_type = genomic RNA
ggcactgactcag

SEQ ID NO: 84 - RNA, 13 nt, Homo sapiens
  misc_feature 1..13: note = Description for SEQ ID NO:84: target regions in region 1+2 of homo sapiens numb exon 9
  source 1..13: mol_type = genomic RNA
gcactgactcagc

SEQ ID NO: 85 - RNA, 13 nt, Homo sapiens
  misc_feature 1..13: note = Description for SEQ ID NO:85: target regions in region 1+2 of homo sapiens numb exon 9
  source 1..13: mol_type = genomic RNA
cactgactcagcc

SEQ ID NO: 86 - RNA, 13 nt, Homo sapiens
  misc_feature 1..13: note = Description for SEQ ID NO:86: target regions in region 1+2 of homo sapiens numb exon 9
  source 1..13: mol_type = genomic RNA
actgactcagcct

SEQ ID NO: 87 - RNA, 13 nt, Homo sapiens
  misc_feature 1..13: note = Description for SEQ ID NO:87: target regions in region 1+2 of homo sapiens numb exon 9
  source 1..13: mol_type = genomic RNA
ctgactcagcctt

SEQ ID NO: 88 - RNA, 13 nt, Homo sapiens
  misc_feature 1..13: note = Description for SEQ ID NO:88: target regions in region 1+2 of homo sapiens numb exon 9
  source 1..13: mol_type = genomic RNA
tgactcagccttc

SEQ ID NO: 89 - RNA, 13 nt, Homo sapiens
  misc_feature 1..13: note = Description for SEQ ID NO:89: target regions in region 1+2 of homo sapiens numb exon 9
  source 1..13: mol_type = genomic RNA
gactcagccttcc

SEQ ID NO: 90 - RNA, 13 nt, Homo sapiens
  misc_feature 1..13: note = Description for SEQ ID NO:90: target regions in region 1+2 of homo sapiens numb exon 9
  source 1..13: mol_type = genomic RNA
actcagccttcca

SEQ ID NO: 91 - RNA, 13 nt, Homo sapiens
  misc_feature 1..13: note = Description for SEQ ID NO:91: target regions in region 1+2 of homo sapiens numb exon 9
  source 1..13: mol_type = genomic RNA
ctcagccttccat

SEQ ID NO: 92 - RNA, 13 nt, Homo sapiens
  misc_feature 1..13: note = Description for SEQ ID NO:92: target regions in region 1+2 of homo sapiens numb exon 9
  source 1..13: mol_type = genomic RNA
tcagccttccatg

SEQ ID NO: 93 - RNA, 13 nt, Homo sapiens
  misc_feature 1..13: note = Description for SEQ ID NO:93: target regions in region 1+2 of homo sapiens numb exon 9
  source 1..13: mol_type = genomic RNA
cagccttccatgt

SEQ ID NO: 94 - RNA, 13 nt, Homo sapiens
  misc_feature 1..13: note = Description for SEQ ID NO:94: target regions in region 1+2 of homo sapiens numb exon 9
  source 1..13: mol_type = genomic RNA
agccttccatgtg

SEQ ID NO: 95 - RNA, 13 nt, Homo sapiens
  misc_feature 1..13: note = Description for SEQ ID NO:95: target regions in region 1+2 of homo sapiens numb exon 9
  source 1..13: mol_type = genomic RNA
gccttccatgtgc

SEQ ID NO: 96 - RNA, 13 nt, Homo sapiens
  misc_feature 1..13: note = Description for SEQ ID NO:96: target regions in region 1+2 of homo sapiens numb exon 9
  source 1..13: mol_type = genomic RNA
ccttccatgtgct

SEQ ID NO: 97 - RNA, 13 nt, Homo sapiens
  misc_feature 1..13: note = Description for SEQ ID NO:97: target regions in region 1+2 of homo sapiens numb exon 9
  source 1..13: mol_type = genomic RNA
cttccatgtgctt

SEQ ID NO: 98 - RNA, 13 nt, Homo sapiens
  misc_feature 1..13: note = Description for SEQ ID NO:98: target regions in region 1+2 of homo sapiens numb exon 9
  source 1..13: mol_type = genomic RNA
ttccatgtgcttg

SEQ ID NO: 99 - RNA, 13 nt, Homo sapiens
  misc_feature 1..13: note = Description for SEQ ID NO:99: target regions in region 1+2 of homo sapiens numb exon 9
  source 1..13: mol_type = genomic RNA
tccatgtgcttgc

SEQ ID NO: 100 - RNA, 13 nt, Homo sapiens
  misc_feature 1..13: note = Description for SEQ ID NO:100: target regions in region 1+2 of homo sapiens numb exon 9
  source 1..13: mol_type = genomic RNA
ccatgtgcttgct

SEQ ID NO: 101 - RNA, 13 nt, Homo sapiens
  misc_feature 1..13: note = Description for SEQ ID NO:101: target regions in region 1+2 of homo sapiens numb exon 9
  source 1..13: mol_type = genomic RNA
catgtgcttgcta

SEQ ID NO: 102 - RNA, 13 nt, Homo sapiens
  misc_feature 1..13: note = Description for SEQ ID NO:102: target regions in region 1+2 of homo sapiens numb exon 9
  source 1..13: mol_type = genomic RNA
atgtgcttgctaa

SEQ ID NO: 103 - RNA, 13 nt, Homo sapiens
  misc_feature 1..13: note = Description for SEQ ID NO:103: target regions in region 1+2 of homo sapiens numb exon 9
  source 1..13: mol_type = genomic RNA
tgtgcttgctaag

SEQ ID NO: 104 - RNA, 13 nt, Homo sapiens
  misc_feature 1..13: note = Description for SEQ ID NO:104: target regions in region 1+2 of homo sapiens numb exon 9
  source 1..13: mol_type = genomic RNA
gtgcttgctaagc

SEQ ID NO: 105 - RNA, 21 nt, Homo sapiens
  misc_feature 1..21: note = Description for SEQ ID NO:105: target regions in region 1+2 of homo sapiens numb exon 9
  source 1..21: mol_type = genomic RNA
ctaatggcactgactcagcct

SEQ ID NO: 106 - RNA, 21 nt, Homo sapiens
  misc_feature 1..21: note = Description for SEQ ID NO:106: target regions in region 1+2 of homo sapiens numb exon 9
  source 1..21: mol_type = genomic RNA
taatggcactgactcagcctt

SEQ ID NO: 107 - RNA, 21 nt, Homo sapiens
  misc_feature 1..21: note = Description for SEQ ID NO:107: target regions in region 1+2 of homo sapiens numb exon 9
  source 1..21: mol_type = genomic RNA
aatggcactgactcagccttc

SEQ ID NO: 108 - RNA, 21 nt, Homo sapiens
  misc_feature 1..21: note = Description for SEQ ID NO:108: target regions in region 1+2 of homo sapiens numb exon 9
  source 1..21: mol_type = genomic RNA
atggcactgactcagccttcc

SEQ ID NO: 109 - RNA, 21 nt, Homo sapiens
  misc_feature 1..21: note = Description for SEQ ID NO:109: target regions in region 1+2 of homo sapiens numb exon 9
  source 1..21: mol_type = genomic RNA
tggcactgactcagccttcca

SEQ ID NO: 110 - RNA, 21 nt, Homo sapiens
  misc_feature 1..21: note = Description for SEQ ID NO:110: target regions in region 1+2 of homo sapiens numb exon 9
  source 1..21: mol_type = genomic RNA
ggcactgactcagccttccat

SEQ ID NO: 111 - RNA, 21 nt, Homo sapiens
  misc_feature 1..21: note = Description for SEQ ID NO:111: target regions in region 1+2 of homo sapiens numb exon 9
  source 1..21: mol_type = genomic RNA
gcactgactcagccttccatg

SEQ ID NO: 112 - RNA, 21 nt, Homo sapiens
  misc_feature 1..21: note = Description for SEQ ID NO:112: target regions in region 1+2 of homo sapiens numb exon 9
  source 1..21: mol_type = genomic RNA
cactgactcagccttccatgt

SEQ ID NO: 113 - RNA, 21 nt, Homo sapiens
  misc_feature 1..21: note = Description for SEQ ID NO:113: target regions in region 1+2 of homo sapiens numb exon 9
  source 1..21: mol_type = genomic RNA
actgactcagccttccatgtg

SEQ ID NO: 114 - RNA, 21 nt, Homo sapiens
  misc_feature 1..21: note = Description for SEQ ID NO:114: target regions in region 1+2 of homo sapiens numb exon 9
  source 1..21: mol_type = genomic RNA
ctgactcagccttccatgtgc

SEQ ID NO: 115 - RNA, 21 nt, Homo sapiens
  misc_feature 1..21: note = Description for SEQ ID NO:115: target regions in region 1+2 of homo sapiens numb exon 9
  source 1..21: mol_type = genomic RNA
tgactcagccttccatgtgct

SEQ ID NO: 116 - RNA, 21 nt, Homo sapiens
  misc_feature 1..21: note = Description for SEQ ID NO:116: target regions in region 1+2 of homo sapiens numb exon 9
  source 1..21: mol_type = genomic RNA
gactcagccttccatgtgctt

SEQ ID NO: 117 - RNA, 21 nt, Homo sapiens
  misc_feature 1..21: note = Description for SEQ ID NO:117: target regions in region 1+2 of homo sapiens numb exon 9
  source 1..21: mol_type = genomic RNA
actcagccttccatgtgcttg

SEQ ID NO: 118 - RNA, 21 nt, Homo sapiens
  misc_feature 1..21: note = Description for SEQ ID NO:118: target regions in region 1+2 of homo sapiens numb exon 9
  source 1..21: mol_type = genomic RNA
ctcagccttccatgtgcttgc

SEQ ID NO: 119 - RNA, 21 nt, Homo sapiens
  misc_feature 1..21: note = Description for SEQ ID NO:119: target regions in region 1+2 of homo sapiens numb exon 9
  source 1..21: mol_type = genomic RNA
tcagccttccatgtgcttgct

SEQ ID NO: 120 - RNA, 21 nt, Homo sapiens
  misc_feature 1..21: note = Description for SEQ ID NO:120: target regions in region 1+2 of homo sapiens numb exon 9
  source 1..21: mol_type = genomic RNA
cagccttccatgtgcttgcta

SEQ ID NO: 121 - RNA, 21 nt, Homo sapiens
  misc_feature 1..21: note = Description for SEQ ID NO:121: target regions in region 1+2 of homo sapiens numb exon 9
  source 1..21: mol_type = genomic RNA
agccttccatgtgcttgctaa

SEQ ID NO: 122 - RNA, 21 nt, Homo sapiens
  misc_feature 1..21: note = Description for SEQ ID NO:122: target regions in region 1+2 of homo sapiens numb exon 9
  source 1..21: mol_type = genomic RNA
gccttccatgtgcttgctaag

SEQ ID NO: 123 - RNA, 21 nt, Homo sapiens
  misc_feature 1..21: note = Description for SEQ ID NO:123: target regions in region 1+2 of homo sapiens numb exon 9
  source 1..21: mol_type = genomic RNA
ccttccatgtgcttgctaagc

SEQ ID NO: 124-159 - skipped (36 entries)

SEQ ID NO: 160 - RNA, 13 nt, Homo sapiens
  misc_feature 1..13: note = Description for SEQ ID NO:160: target regions in region 4+5 of homo sapiens numb exon 9
  source 1..13: mol_type = genomic RNA
ccgtagcaatgcc

SEQ ID NO: 161 - RNA, 13 nt, Homo sapiens
  misc_feature 1..13: note = Description for SEQ ID NO:161: target regions in region 4+5 of homo sapiens numb exon 9
  source 1..13: mol_type = genomic RNA
cgtagcaatgcct

SEQ ID NO: 162 - RNA, 13 nt, Homo sapiens
  misc_feature 1..13: note = Description for SEQ ID NO:162: target regions in region 4+5 of homo sapiens numb exon 9
  source 1..13: mol_type = genomic RNA
gtagcaatgcctg

SEQ ID NO: 163 - RNA, 13 nt, Homo sapiens
  misc_feature 1..13: note = Description for SEQ ID NO:163: target regions in region 4+5 of homo sapiens numb exon 9
  source 1..13: mol_type = genomic RNA
tagcaatgcctgt

SEQ ID NO: 164 - RNA, 13 nt, Homo sapiens
  misc_feature 1..13: note = Description for SEQ ID NO:164: target regions in region 4+5 of homo sapiens numb exon 9
  source 1..13: mol_type = genomic RNA
agcaatgcctgtg

SEQ ID NO: 165 - RNA, 13 nt, Homo sapiens
  misc_feature 1..13: note = Description for SEQ ID NO:165: target regions in region 4+5 of homo sapiens numb exon 9
  source 1..13: mol_type = genomic RNA
gcaatgcctgtgc

SEQ ID NO: 166 - RNA, 13 nt, Homo sapiens
  misc_feature 1..13: note = Description for SEQ ID NO:166: target regions in region 4+5 of homo sapiens numb exon 9
  source 1..13: mol_type = genomic RNA
caatgcctgtgcg

SEQ ID NO: 167 - RNA, 13 nt, Homo sapiens
  misc_feature 1..13: note = Description for SEQ ID NO:167: target regions in region 4+5 of homo sapiens numb exon 9
  source 1..13: mol_type = genomic RNA
aatgcctgtgcgt

SEQ ID NO: 168 - RNA, 13 nt, Homo sapiens
  misc_feature 1..13: note = Description for SEQ ID NO:168: target regions in region 4+5 of homo sapiens numb exon 9
  source 1..13: mol_type = genomic RNA
atgcctgtgcgtg

SEQ ID NO: 169 - RNA, 13 nt, Homo sapiens
  misc_feature 1..13: note = Description for SEQ ID NO:169: target regions in region 4+5 of homo sapiens numb exon 9
  source 1..13: mol_type = genomic RNA
tgcctgtgcgtga

SEQ ID NO: 170 - RNA, 13 nt, Homo sapiens
  misc_feature 1..13: note = Description for SEQ ID NO:170: target regions in region 4+5 of homo sapiens numb exon 9
  source 1..13: mol_type = genomic RNA
gcctgtgcgtgaa

SEQ ID NO: 171 - RNA, 13 nt, Homo sapiens
  misc_feature 1..13: note = Description for SEQ ID NO:171: target regions in region 4+5 of homo sapiens numb exon 9
  source 1..13: mol_type = genomic RNA
cctgtgcgtgaaa

SEQ ID NO: 172 - RNA, 13 nt, Homo sapiens
  misc_feature 1..13: note = Description for SEQ ID NO:172: target regions in region 4+5 of homo sapiens numb exon 9
  source 1..13: mol_type = genomic RNA
ctgtgcgtgaaac

SEQ ID NO: 173 - RNA, 13 nt, Homo sapiens
  misc_feature 1..13: note = Description for SEQ ID NO:173: target regions in region 4+5 of homo sapiens numb exon 9
  source 1..13: mol_type = genomic RNA
tgtgcgtgaaacc

SEQ ID NO: 174 - RNA, 13 nt, Homo sapiens
  misc_feature 1..13: note = Description for SEQ ID NO:174: target regions in region 4+5 of homo sapiens numb exon 9
  source 1..13: mol_type = genomic RNA
gtgcgtgaaacca

SEQ ID NO: 175 - RNA, 13 nt, Homo sapiens
  misc_feature 1..13: note = Description for SEQ ID NO:175: target regions in region 4+5 of homo sapiens numb exon 9
  source 1..13: mol_type = genomic RNA
tgcgtgaaaccaa

SEQ ID NO: 176 - RNA, 13 nt, Homo sapiens
  misc_feature 1..13: note = Description for SEQ ID NO:176: target regions in region 4+5 of homo sapiens numb exon 9
  source 1..13: mol_type = genomic RNA
gcgtgaaaccaac

SEQ ID NO: 177 - RNA, 13 nt, Homo sapiens
  misc_feature 1..13: note = Description for SEQ ID NO:177: target regions in region 4+5 of homo sapiens numb exon 9
  source 1..13: mol_type = genomic RNA
cgtgaaaccaacc

SEQ ID NO: 178 - RNA, 13 nt, Homo sapiens
  misc_feature 1..13: note = Description for SEQ ID NO:178: target regions in region 4+5 of homo sapiens numb exon 9
  source 1..13: mol_type = genomic RNA
gtgaaaccaaccc

SEQ ID NO: 179 - RNA, 13 nt, Homo sapiens
  misc_feature 1..13: note = Description for SEQ ID NO:179: target regions in region 4+5 of homo sapiens numb exon 9
  source 1..13: mol_type = genomic RNA
tgaaaccaaccct

SEQ ID NO: 180 - RNA, 13 nt, Homo sapiens
  misc_feature 1..13: note = Description for SEQ ID NO:180: target regions in region 4+5 of homo sapiens numb exon 9
  source 1..13: mol_type = genomic RNA
gaaaccaaccctt

SEQ ID NO: 181 - RNA, 13 nt, Homo sapiens
  misc_feature 1..13: note = Description for SEQ ID NO:181: target regions in region 4+5 of homo sapiens numb exon 9
  source 1..13: mol_type = genomic RNA
aaaccaacccttg

SEQ ID NO: 182 - RNA, 13 nt, Homo sapiens
  misc_feature 1..13: note = Description for SEQ ID NO:182: target regions in region 4+5 of homo sapiens numb exon 9
  source 1..13: mol_type = genomic RNA
aaccaacccttgg

SEQ ID NO: 183 - RNA, 13 nt, Homo sapiens
  misc_feature 1..13: note = Description for SEQ ID NO:183: target regions in region 4+5 of homo sapiens numb exon 9
  source 1..13: mol_type = genomic RNA
accaacccttggg

SEQ ID NO: 184 - RNA, 13 nt, Homo sapiens
  misc_feature 1..13: note = Description for SEQ ID NO:184: target regions in region 4+5 of homo sapiens numb exon 9
  source 1..13: mol_type = genomic RNA
ccaacccttgggc

SEQ ID NO: 185 - RNA, 13 nt, Homo sapiens
  misc_feature 1..13: note = Description for SEQ ID NO:185: target regions in region 4+5 of homo sapiens numb exon 9
  source 1..13: mol_type = genomic RNA
caacccttgggcc

SEQ ID NO: 186 - RNA, 13 nt, Homo sapiens
  misc_feature 1..13: note = Description for SEQ ID NO:186: target regions in region 4+5 of homo sapiens numb exon 9
  source 1..13: mol_type = genomic RNA
aacccttgggccc

SEQ ID NO: 187 - RNA, 13 nt, Homo sapiens
  misc_feature 1..13: note = Description for SEQ ID NO:187: target regions in region 4+5 of homo sapiens numb exon 9
  source 1..13: mol_type = genomic RNA
acccttgggccca

SEQ ID NO: 188 - RNA, 13 nt, Homo sapiens
  misc_feature 1..13: note = Description for SEQ ID NO:188: target regions in region 4+5 of homo sapiens numb exon 9
  source 1..13: mol_type = genomic RNA
cccttgggcccat

SEQ ID NO: 189 - RNA, 13 nt, Homo sapiens
  misc_feature 1..13: note = Description for SEQ ID NO:189: target regions in region 4+5 of homo sapiens numb exon 9
  source 1..13: mol_type = genomic RNA
ccttgggcccatg

SEQ ID NO: 190 - RNA, 21 nt, Homo sapiens
  misc_feature 1..21: note = Description for SEQ ID NO:190: target regions in region 4+5 of homo sapiens numb exon 9
  source 1..21: mol_type = genomic RNA
ccgtagcaatgcctgtgcgtg

SEQ ID NO: 191 - RNA, 21 nt, Homo sapiens
  misc_feature 1..21: note = Description for SEQ ID NO:191: target regions in region 4+5 of homo sapiens numb exon 9
  source 1..21: mol_type = genomic RNA
cgtagcaatgcctgtgcgtga

SEQ ID NO: 192 - RNA, 21 nt, Homo sapiens
  misc_feature 1..21: note = Description for SEQ ID NO:192: target regions in region 4+5 of homo sapiens numb exon 9
  source 1..21: mol_type = genomic RNA
gtagcaatgcctgtgcgtgaa

SEQ ID NO: 193 - RNA, 21 nt, Homo sapiens
  misc_feature 1..21: note = Description for SEQ ID NO:193: target regions in region 4+5 of homo sapiens numb exon 9
  source 1..21: mol_type = genomic RNA
tagcaatgcctgtgcgtgaaa

SEQ ID NO: 194 - RNA, 21 nt, Homo sapiens
  misc_feature 1..21: note = Description for SEQ ID NO:194: target regions in region 4+5 of homo sapiens numb exon 9
  source 1..21: mol_type = genomic RNA
agcaatgcctgtgcgtgaaac

SEQ ID NO: 195 - RNA, 21 nt, Homo sapiens
  misc_feature 1..21: note = Description for SEQ ID NO:195: target regions in region 4+5 of homo sapiens numb exon 9
  source 1..21: mol_type = genomic RNA
gcaatgcctgtgcgtgaaacc

SEQ ID NO: 196 - RNA, 21 nt, Homo sapiens
  misc_feature 1..21: note = Description for SEQ ID NO:196: target regions in region 4+5 of homo sapiens numb exon 9
  source 1..21: mol_type = genomic RNA
caatgcctgtgcgtgaaacca

SEQ ID NO: 197 - RNA, 21 nt, Homo sapiens
  misc_feature 1..21: note = Description for SEQ ID NO:197: target regions in region 4+5 of homo sapiens numb exon 9
  source 1..21: mol_type = genomic RNA
aatgcctgtgcgtgaaaccaa

SEQ ID NO: 198 - RNA, 21 nt, Homo sapiens
  misc_feature 1..21: note = Description for SEQ ID NO:198: target regions in region 4+5 of homo sapiens numb exon 9
  source 1..21: mol_type = genomic RNA
atgcctgtgcgtgaaaccaac

SEQ ID NO: 199 - RNA, 21 nt, Homo sapiens
  misc_feature 1..21: note = Description for SEQ ID NO:199: target regions in region 4+5 of homo sapiens numb exon 9
  source 1..21: mol_type = genomic RNA
tgcctgtgcgtgaaaccaacc

SEQ ID NO: 200 - RNA, 21 nt, Homo sapiens
  misc_feature 1..21: note = Description for SEQ ID NO:200: target regions in region 4+5 of homo sapiens numb exon 9
  source 1..21: mol_type = genomic RNA
gcctgtgcgtgaaaccaaccc

SEQ ID NO: 201 - RNA, 21 nt, Homo sapiens
  misc_feature 1..21: note = Description for SEQ ID NO:201: target regions in region 4+5 of homo sapiens numb exon 9
  source 1..21: mol_type = genomic RNA
cctgtgcgtgaaaccaaccct

SEQ ID NO: 202 - RNA, 21 nt, Homo sapiens
  misc_feature 1..21: note = Description for SEQ ID NO:202: target regions in region 4+5 of homo sapiens numb exon 9
  source 1..21: mol_type = genomic RNA
ctgtgcgtgaaaccaaccctt

SEQ ID NO: 203 - RNA, 21 nt, Homo sapiens
  misc_feature 1..21: note = Description for SEQ ID NO:203: target regions in region 4+5 of homo sapiens numb exon 9
  source 1..21: mol_type = genomic RNA
tgtgcgtgaaaccaacccttg

SEQ ID NO: 204 - RNA, 21 nt, Homo sapiens
  misc_feature 1..21: note = Description for SEQ ID NO:204: target regions in region 4+5 of homo sapiens numb exon 9
  source 1..21: mol_type = genomic RNA
gtgcgtgaaaccaacccttgg

SEQ ID NO: 205 - RNA, 21 nt, Homo sapiens
  misc_feature 1..21: note = Description for SEQ ID NO:205: target regions in region 4+5 of homo sapiens numb exon 9
  source 1..21: mol_type = genomic RNA
tgcgtgaaaccaacccttggg

SEQ ID NO: 206 - RNA, 21 nt, Homo sapiens
  misc_feature 1..21: note = Description for SEQ ID NO:206: target regions in region 4+5 of homo sapiens numb exon 9
  source 1..21: mol_type = genomic RNA
gcgtgaaaccaacccttgggc

SEQ ID NO: 207 - RNA, 21 nt, Homo sapiens
  misc_feature 1..21: note = Description for SEQ ID NO:207: target regions in region 4+5 of homo sapiens numb exon 9
  source 1..21: mol_type = genomic RNA
cgtgaaaccaacccttgggcc

SEQ ID NO: 208 - RNA, 21 nt, Homo sapiens
  misc_feature 1..21: note = Description for SEQ ID NO:208: target regions in region 4+5 of homo sapiens numb exon 9
  source 1..21: mol_type = genomic RNA
gtgaaaccaacccttgggccc

SEQ ID NO: 209 - RNA, 21 nt, Homo sapiens
  misc_feature 1..21: note = Description for SEQ ID NO:209: target regions in region 4+5 of homo sapiens numb exon 9
  source 1..21: mol_type = genomic RNA
tgaaaccaacccttgggccca

SEQ ID NO: 210 - RNA, 21 nt, Homo sapiens
  misc_feature 1..21: note = Description for SEQ ID NO:210: target regions in region 4+5 of homo sapiens numb exon 9
  source 1..21: mol_type = genomic RNA
gaaaccaacccttgggcccat

SEQ ID NO: 211 - RNA, 21 nt, Homo sapiens
  misc_feature 1..21: note = Description for SEQ ID NO:211: target regions in region 4+5 of homo sapiens numb exon 9
  source 1..21: mol_type = genomic RNA
aaaccaacccttgggcccatg

SEQ ID NO: 212-247 - skipped (36 entries)

SEQ ID NO: 248 - RNA, 13 nt, Homo sapiens
  misc_feature 1..13: note = Description for SEQ ID NO:248: target regions in region 6+7 of homo sapiens numb exon 9
  source 1..13: mol_type = genomic RNA
cccctgatgctgc

SEQ ID NO: 249 - RNA, 13 nt, Homo sapiens
  misc_feature 1..13: note = Description for SEQ ID NO:249: target regions in region 6+7 of homo sapiens numb exon 9
  source 1..13: mol_type = genomic RNA
ccctgatgctgct

SEQ ID NO: 250 - RNA, 13 nt, Homo sapiens
  misc_feature 1..13: note = Description for SEQ ID NO:250: target regions in region 6+7 of homo sapiens numb exon 9
  source 1..13: mol_type = genomic RNA
cctgatgctgcta

SEQ ID NO: 251 - RNA, 13 nt, Homo sapiens
  misc_feature 1..13: note = Description for SEQ ID NO:251: target regions in region 6+7 of homo sapiens numb exon 9
  source 1..13: mol_type = genomic RNA
ctgatgctgctaa

SEQ ID NO: 252 - RNA, 13 nt, Homo sapiens
  misc_feature 1..13: note = Description for SEQ ID NO:252: target regions in region 6+7 of homo sapiens numb exon 9
  source 1..13: mol_type = genomic RNA
tgatgctgctaac

SEQ ID NO: 253 - RNA, 13 nt, Homo sapiens
  misc_feature 1..13: note = Description for SEQ ID NO:253: target regions in region 6+7 of homo sapiens numb exon 9
  source 1..13: mol_type = genomic RNA
gatgctgctaaca

SEQ ID NO: 254 - RNA, 13 nt, Homo sapiens
  misc_feature 1..13: note = Description for SEQ ID NO:254: target regions in region 6+7 of homo sapiens numb exon 9
  source 1..13: mol_type = genomic RNA
atgctgctaacaa

SEQ ID NO: 255 - RNA, 13 nt, Homo sapiens
  misc_feature 1..13: note = Description for SEQ ID NO:255: target regions in region 6+7 of homo sapiens numb exon 9
  source 1..13: mol_type = genomic RNA
tgctgctaacaag

SEQ ID NO: 256 - RNA, 13 nt, Homo sapiens
  misc_feature 1..13: note = Description for SEQ ID NO:256: target regions in region 6+7 of homo sapiens numb exon 9
  source 1..13: mol_type = genomic RNA
gctgctaacaagg

SEQ ID NO: 257 - RNA, 13 nt, Homo sapiens
  misc_feature 1..13: note = Description for SEQ ID NO:257: target regions in region 6+7 of homo sapiens numb exon 9
  source 1..13: mol_type = genomic RNA
ctgctaacaagga

SEQ ID NO: 258 - RNA, 13 nt, Homo sapiens
  misc_feature 1..13: note = Description for SEQ ID NO:258: target regions in region 6+7 of homo sapiens numb exon 9
  source 1..13: mol_type = genomic RNA
tgctaacaaggaa

SEQ ID NO: 259 - RNA, 13 nt, Homo sapiens
  misc_feature 1..13: note = Description for SEQ ID NO:259: target regions in region 6+7 of homo sapiens numb exon 9
  source 1..13: mol_type = genomic RNA
gctaacaaggaaa

SEQ ID NO: 260 - RNA, 13 nt, Homo sapiens
  misc_feature 1..13: note = Description for SEQ ID NO:260: target regions in region 6+7 of homo sapiens numb exon 9
  source 1..13: mol_type = genomic RNA
ctaacaaggaaat

SEQ ID NO: 261 - RNA, 13 nt, Homo sapiens
  misc_feature 1..13: note = Description for SEQ ID NO:261: target regions in region 6+7 of homo sapiens numb exon 9
  source 1..13: mol_type = genomic RNA
taacaaggaaatt

SEQ ID NO: 262 - RNA, 13 nt, Homo sapiens
  misc_feature 1..13: note = Description for SEQ ID NO:262: target regions in region 6+7 of homo sapiens numb exon 9
  source 1..13: mol_type = genomic RNA
aacaaggaaattg

SEQ ID NO: 263 - RNA, 13 nt, Homo sapiens
  misc_feature 1..13: note = Description for SEQ ID NO:263: target regions in region 6+7 of homo sapiens numb exon 9
  source 1..13: mol_type = genomic RNA
acaaggaaattgc

SEQ ID NO: 264 - RNA, 13 nt, Homo sapiens
  misc_feature 1..13: note = Description for SEQ ID NO:264: target regions in region 6+7 of homo sapiens numb exon 9
  source 1..13: mol_type = genomic RNA
caaggaaattgca

SEQ ID NO: 265 - RNA, 13 nt, Homo sapiens
  misc_feature 1..13: note = Description for SEQ ID NO:265: target regions in region 6+7 of homo sapiens numb exon 9
  source 1..13: mol_type = genomic RNA
aaggaaattgcag

SEQ ID NO: 266 - RNA, 13 nt, Homo sapiens
  misc_feature 1..13: note = Description for SEQ ID NO:266: target regions in region 6+7 of homo sapiens numb exon 9
  source 1..13: mol_type = genomic RNA
aggaaattgcagc

SEQ ID NO: 267 - RNA, 13 nt, Homo sapiens
  misc_feature 1..13: note = Description for SEQ ID NO:267: target regions in region 6+7 of homo sapiens numb exon 9
  source 1..13: mol_type = genomic RNA
ggaaattgcagcc

SEQ ID NO: 268 - RNA, 13 nt, Homo sapiens
  misc_feature 1..13: note = Description for SEQ ID NO:268: target regions in region 6+7 of homo sapiens numb exon 9
  source 1..13: mol_type = genomic RNA
gaaattgcagcca

SEQ ID NO: 269 - RNA, 13 nt, Homo sapiens
  misc_feature 1..13: note = Description for SEQ ID NO:269: target regions in region 6+7 of homo sapiens numb exon 9
  source 1..13: mol_type = genomic RNA
aaattgcagccac

SEQ ID NO: 270 - RNA, 13 nt, Homo sapiens
  misc_feature 1..13: note = Description for SEQ ID NO:270: target regions in region 6+7 of homo sapiens numb exon 9
  source 1..13: mol_type = genomic RNA
aattgcagccaca

SEQ ID NO: 271 - RNA, 13 nt, Homo sapiens
  misc_feature 1..13: note = Description for SEQ ID NO:271: target regions in region 6+7 of homo sapiens numb exon 9
  source 1..13: mol_type = genomic RNA
attgcagccacat

SEQ ID NO: 272 - RNA, 13 nt, Homo sapiens
  misc_feature 1..13: note = Description for SEQ ID NO:272: target regions in region 6+7 of homo sapiens numb exon 9
  source 1..13: mol_type = genomic RNA
ttgcagccacatg

SEQ ID NO: 273 - RNA, 13 nt, Homo sapiens
  misc_feature 1..13: note = Description for SEQ ID NO:273: target regions in region 6+7 of homo sapiens numb exon 9
  source 1..13: mol_type = genomic RNA
tgcagccacatgt

SEQ ID NO: 274 - RNA, 13 nt, Homo sapiens
  misc_feature 1..13: note = Description for SEQ ID NO:274: target regions in region 6+7 of homo sapiens numb exon 9
  source 1..13: mol_type = genomic RNA
gcagccacatgtt

SEQ ID NO: 275 - RNA, 13 nt, Homo sapiens
  misc_feature 1..13: note = Description for SEQ ID NO:275: target regions in region 6+7 of homo sapiens numb exon 9
  source 1..13: mol_type = genomic RNA
cagccacatgttc

SEQ ID NO: 276 - RNA, 13 nt, Homo sapiens
  misc_feature 1..13: note = Description for SEQ ID NO:276: target regions in region 6+7 of homo sapiens numb exon 9
  source 1..13: mol_type = genomic RNA
agccacatgttcg

SEQ ID NO: 277 - RNA, 13 nt, Homo sapiens
  misc_feature 1..13: note = Description for SEQ ID NO:277: target regions in region 6+7 of homo sapiens numb exon 9
  source 1..13: mol_type = genomic RNA
gccacatgttcgg

SEQ ID NO: 278 - RNA, 21 nt, Homo sapiens
  misc_feature 1..21: note = Description for SEQ ID NO:278: target regions in region 6+7 of homo sapiens numb exon 9
  source 1..21: mol_type = genomic RNA
cccctgatgctgctaacaagg

SEQ ID NO: 279 - RNA, 21 nt, Homo sapiens
  misc_feature 1..21: note = Description for SEQ ID NO:279: target regions in region 6+7 of homo sapiens numb exon 9
  source 1..21: mol_type = genomic RNA
ccctgatgctgctaacaagga

SEQ ID NO: 280 - RNA, 21 nt, Homo sapiens
  misc_feature 1..21: note = Description for SEQ ID NO:280: target regions in region 6+7 of homo sapiens numb exon 9
  source 1..21: mol_type = genomic RNA
cctgatgctgctaacaaggaa

SEQ ID NO: 281 - RNA, 21 nt, Homo sapiens
  misc_feature 1..21: note = Description for SEQ ID NO:281: target regions in region 6+7 of homo sapiens numb exon 9
  source 1..21: mol_type = genomic RNA
ctgatgctgctaacaaggaaa

SEQ ID NO: 282 - RNA, 21 nt, Homo sapiens
  misc_feature 1..21: note = Description for SEQ ID NO:282: target regions in region 6+7 of homo sapiens numb exon 9
  source 1..21: mol_type = genomic RNA
tgatgctgctaacaaggaaat

SEQ ID NO: 283 - RNA, 21 nt, Homo sapiens
  misc_feature 1..21: note = Description for SEQ ID NO:283: target regions in region 6+7 of homo sapiens numb exon 9
  source 1..21: mol_type = genomic RNA
gatgctgctaacaaggaaatt

SEQ ID NO: 284 - RNA, 21 nt, Homo sapiens
  misc_feature 1..21: note = Description for SEQ ID NO:284: target regions in region 6+7 of homo sapiens numb exon 9
  source 1..21: mol_type = genomic RNA
atgctgctaacaaggaaattg

SEQ ID NO: 285 - RNA, 21 nt, Homo sapiens
  misc_feature 1..21: note = Description for SEQ ID NO:285: target regions in region 6+7 of homo sapiens numb exon 9
  source 1..21: mol_type = genomic RNA
tgctgctaacaaggaaattgc

SEQ ID NO: 286 - RNA, 21 nt, Homo sapiens
  misc_feature 1..21: note = Description for SEQ ID NO:286: target regions in region 6+7 of homo sapiens numb exon 9
  source 1..21: mol_type = genomic RNA
gctgctaacaaggaaattgca

SEQ ID NO: 287 - RNA, 21 nt, Homo sapiens
  misc_feature 1..21: note = Description for SEQ ID NO:287: target regions in region 6+7 of homo sapiens numb exon 9
  source 1..21: mol_type = genomic RNA
ctgctaacaaggaaattgcag

SEQ ID NO: 288 - RNA, 21 nt, Homo sapiens
  misc_feature 1..21: note = Description for SEQ ID NO:288: target regions in region 6+7 of homo sapiens numb exon 9
  source 1..21: mol_type = genomic RNA
tgctaacaaggaaattgcagc

SEQ ID NO: 289 - RNA, 21 nt, Homo sapiens
  misc_feature 1..21: note = Description for SEQ ID NO:289: target regions in region 6+7 of homo sapiens numb exon 9
  source 1..21: mol_type = genomic RNA
gctaacaaggaaattgcagcc

SEQ ID NO: 290 - RNA, 21 nt, Homo sapiens
  misc_feature 1..21: note = Description for SEQ ID NO:290: target regions in region 6+7 of homo sapiens numb exon 9
  source 1..21: mol_type = genomic RNA
ctaacaaggaaattgcagcca

SEQ ID NO: 291 - RNA, 21 nt, Homo sapiens
  misc_feature 1..21: note = Description for SEQ ID NO:291: target regions in region 6+7 of homo sapiens numb exon 9
  source 1..21: mol_type = genomic RNA
taacaaggaaattgcagccac

SEQ ID NO: 292 - RNA, 21 nt, Homo sapiens
  misc_feature 1..21: note = Description for SEQ ID NO:292: target regions in region 6+7 of homo sapiens numb exon 9
  source 1..21: mol_type = genomic RNA
aacaaggaaattgcagccaca

SEQ ID NO: 293 - RNA, 21 nt, Homo sapiens
  misc_feature 1..21: note = Description for SEQ ID NO:293: target regions in region 6+7 of homo sapiens numb exon 9
  source 1..21: mol_type = genomic RNA
acaaggaaattgcagccacat

SEQ ID NO: 294 - RNA, 21 nt, Homo sapiens
  misc_feature 1..21: note = Description for SEQ ID NO:294: target regions in region 6+7 of homo sapiens numb exon 9
  source 1..21: mol_type = genomic RNA
caaggaaattgcagccacatg

SEQ ID NO: 295 - RNA, 21 nt, Homo sapiens
  misc_feature 1..21: note = Description for SEQ ID NO:295: target regions in region 6+7 of homo sapiens numb exon 9
  source 1..21: mol_type = genomic RNA
aaggaaattgcagccacatgt

SEQ ID NO: 296 - RNA, 21 nt, Homo sapiens
  misc_feature 1..21: note = Description for SEQ ID NO:296: target regions in region 6+7 of homo sapiens numb exon 9
  source 1..21: mol_type = genomic RNA
aggaaattgcagccacatgtt

SEQ ID NO: 297 - RNA, 21 nt, Homo sapiens
  misc_feature 1..21: note = Description for SEQ ID NO:297: target regions in region 6+7 of homo sapiens numb exon 9
  source 1..21: mol_type = genomic RNA
ggaaattgcagccacatgttc

SEQ ID NO: 298 - RNA, 21 nt, Homo sapiens
  misc_feature 1..21: note = Description for SEQ ID NO:298: target regions in region 6+7 of homo sapiens numb exon 9
  source 1..21: mol_type = genomic RNA
gaaattgcagccacatgttcg

SEQ ID NO: 299 - RNA, 21 nt, Homo sapiens
  misc_feature 1..21: note = Description for SEQ ID NO:299: target regions in region 6+7 of homo sapiens numb exon 9
  source 1..21: mol_type = genomic RNA
aaattgcagccacatgttcgg

SEQ ID NO: 300 - DNA, 11 bp, Homo sapiens
  misc_feature 1..11: note = Description for SEQ ID NO:Potential binding site of SF1/BBP in NUMB exon 9
  source 1..11: mol_type = genomic DNA
ggcactgactc

SEQ ID NO: 301 - DNA, 11 bp, synthetic construct
  misc_feature 1..11: note = Description for SEQ ID NO:RG6-NUMB minigene WT
  source 1..11: mol_type = other DNA
ggcactgactc

SEQ ID NO: 302 - DNA, 12 bp, synthetic construct
  misc_feature 1..12: note = Description for SEQ ID NO:RG6-NUMB minigene Mut3
  source 1..12: mol_type = other DNA
ggcactcacctc

SEQ ID NO: 303 - DNA, 11 bp, synthetic construct
  misc_feature 1..11: note = Description for SEQ ID NO:RG6-NUMB minigene Mut 4
  source 1..11: mol_type = other DNA
ggcaccgactc

SEQ ID NO: 304 - DNA, 12 bp, synthetic construct
  misc_feature 1..12: note = Description for SEQ ID NO:RG6-NUMB minigene Mut 1
  source 1..12: mol_type = other DNA
ggtactgacctc

SEQ ID NO: 305 - RNA, 50 nt, Homo sapiens
  misc_feature 1..50: note = Description for SEQ ID NO:Region 1+2+ 2-3 of Homo sapiens Numb exon 9 (targeted by by AON1 SEQ ID NO: 12; AON2 SEQ ID NO: 13; AON1-2 SEQ ID NO: 19; and AON2-3 SEQ ID NO:20)
  source 1..50: mol_type = genomic RNA
ctaatggcactgactcagccttccatgtgcttgctaagccagcccatact

SEQ ID NO: 306-316 - skipped (11 entries)

SEQ ID NO: 317 - RNA, 13 nt, Homo sapiens
  misc_feature 1..13: note = Description for SEQ ID NO:317: target regions in region 1+2+2-3 of homo sapiens numb exon 9
  source 1..13: mol_type = genomic RNA
tgcttgctaagcc

SEQ ID NO: 318 - RNA, 13 nt, Homo sapiens
  misc_feature 1..13: note = Description for SEQ ID NO:318: target regions in region 1+2+2-3 of homo sapiens numb exon 9
  source 1..13: mol_type = genomic RNA
gcttgctaagcca

SEQ ID NO: 319 - RNA, 13 nt, Homo sapiens
  misc_feature 1..13: note = Description for SEQ ID NO:319: target regions in region 1+2+2-3 of homo sapiens numb exon 9
  source 1..13: mol_type = genomic RNA
cttgctaagccag

SEQ ID NO: 320 - RNA, 13 nt, Homo sapiens
  misc_feature 1..13: note = Description for SEQ ID NO:320: target regions in region 1+2+2-3 of homo sapiens numb exon 9
  source 1..13: mol_type = genomic RNA
ttgctaagccagc

SEQ ID NO: 321 - RNA, 13 nt, Homo sapiens
  misc_feature 1..13: note = Description for SEQ ID NO:321: target regions in region 1+2+2-3 of homo sapiens numb exon 9
  source 1..13: mol_type = genomic RNA
tgctaagccagcc

SEQ ID NO: 322 - RNA, 13 nt, Homo sapiens
  misc_feature 1..13: note = Description for SEQ ID NO:322: target regions in region 1+2+2-3 of homo sapiens numb exon 9
  source 1..13: mol_type = genomic RNA
gctaagccagccc

SEQ ID NO: 323 - RNA, 13 nt, Homo sapiens
  misc_feature 1..13: note = Description for SEQ ID NO:323: target regions in region 1+2+2-3 of homo sapiens numb exon 9
  source 1..13: mol_type = genomic RNA
ctaagccagccca

SEQ ID NO: 324 - RNA, 13 nt, Homo sapiens
  misc_feature 1..13: note = Description for SEQ ID NO:324: target regions in region 1+2+2-3 of homo sapiens numb exon 9
  source 1..13: mol_type = genomic RNA
taagccagcccat

SEQ ID NO: 325 - RNA, 13 nt, Homo sapiens
  misc_feature 1..13: note = Description for SEQ ID NO:325: target regions in region 1+2+2-3 of homo sapiens numb exon 9
  source 1..13: mol_type = genomic RNA
aagccagcccata

SEQ ID NO: 326 - RNA, 13 nt, Homo sapiens
  misc_feature 1..13: note = Description for SEQ ID NO:326: target regions in region 1+2+2-3 of homo sapiens numb exon 9
  source 1..13: mol_type = genomic RNA
agccagcccatac

SEQ ID NO: 327 - RNA, 13 nt, Homo sapiens
  misc_feature 1..13: note = Description for SEQ ID NO:327: target regions in region 1+2+2-3 of homo sapiens numb exon 9
  source 1..13: mol_type = genomic RNA
gccagcccatact

SEQ ID NO: 328 - RNA, 21 nt, Homo sapiens
  misc_feature 1..21: note = Description for SEQ ID NO:328: target regions in region 1+2+2-3 of homo sapiens numb exon 9
  source 1..21: mol_type = genomic RNA
cttccatgtgcttgctaagcc

SEQ ID NO: 329 - RNA, 21 nt, Homo sapiens
  misc_feature 1..21: note = Description for SEQ ID NO:329: target regions in region 1+2+2-3 of homo sapiens numb exon 9
  source 1..21: mol_type = genomic RNA
ttccatgtgcttgctaagcca

SEQ ID NO: 330 - RNA, 21 nt, Homo sapiens
  misc_feature 1..21: note = Description for SEQ ID NO:330: target regions in region 1+2+2-3 of homo sapiens numb exon 9
  source 1..21: mol_type = genomic RNA
tccatgtgcttgctaagccag

SEQ ID NO: 331 - RNA, 21 nt, Homo sapiens
  misc_feature 1..21: note = Description for SEQ ID NO:331: target regions in region 1+2+2-3 of homo sapiens numb exon 9
  source 1..21: mol_type = genomic RNA
ccatgtgcttgctaagccagc

SEQ ID NO: 332 - RNA, 21 nt, Homo sapiens
  misc_feature 1..21: note = Description for SEQ ID NO:332: target regions in region 1+2+2-3 of homo sapiens numb exon 9
  source 1..21: mol_type = genomic RNA
catgtgcttgctaagccagcc

SEQ ID NO: 333 - RNA, 21 nt, Homo sapiens
  misc_feature 1..21: note = Description for SEQ ID NO:333: target regions in region 1+2+2-3 of homo sapiens numb exon 9
  source 1..21: mol_type = genomic RNA
atgtgcttgctaagccagccc

SEQ ID NO: 334 - RNA, 21 nt, Homo sapiens
  misc_feature 1..21: note = Description for SEQ ID NO:334: target regions in region 1+2+2-3 of homo sapiens numb exon 9
  source 1..21: mol_type = genomic RNA
tgtgcttgctaagccagccca

SEQ ID NO: 335 - RNA, 21 nt, Homo sapiens
  misc_feature 1..21: note = Description for SEQ ID NO:335: target regions in region 1+2+2-3 of homo sapiens numb exon 9
  source 1..21: mol_type = genomic RNA
gtgcttgctaagccagcccat

SEQ ID NO: 336 - RNA, 21 nt, Homo sapiens
  misc_feature 1..21: note = Description for SEQ ID NO:336: target regions in region 1+2+2-3 of homo sapiens numb exon 9
  source 1..21: mol_type = genomic RNA
tgcttgctaagccagcccata

SEQ ID NO: 337 - RNA, 21 nt, Homo sapiens
  misc_feature 1..21: note = Description for SEQ ID NO:337: target regions in region 1+2+2-3 of homo sapiens numb exon 9
  source 1..21: mol_type = genomic RNA
gcttgctaagccagcccatac

SEQ ID NO: 338 - RNA, 21 nt, Homo sapiens
  misc_feature 1..21: note = Description for SEQ ID NO:338: target regions in region 1+2+2-3 of homo sapiens numb exon 9
  source 1..21: mol_type = genomic RNA
cttgctaagccagcccatact

SEQ ID NO: 339 - RNA, 14 nt, Homo sapiens
  misc_feature 1..14: note = Description for SEQ ID NO:339: Antisense oligonucleotide targeting Region 1 of Homo sapiens Numb exon 9 14 nt long, targeting second part of region defined by SEQ ID NO:44
  source 1..14: mol_type = genomic RNA
aggctgagtcagtg

SEQ ID NO: 340 - RNA, 14 nt, Homo sapiens
  misc_feature 1..14: note = Description for SEQ ID NO:340: Antisense oligonucleotide targeting Region 1 of Homo sapiens Numb exon 9 14 nt long, targeting firstpart of region defined by SEQ ID NO:44
  source 1..14: mol_type = genomic RNA
gtcagtgccattag

SEQ ID NO: 341 - RNA, 14 nt, Homo sapiens
  misc_feature 1..14: note = Description for SEQ ID NO:341: Homo sapiens Numb exon 9 sequence targeted by antisense oligonucleotide of SEQ ID NO: 339
  source 1..14: mol_type = genomic RNA
cactgactcagcct

SEQ ID NO: 342 - RNA, 14 nt, Homo sapiens
  misc_feature 1..14: note = Description for SEQ ID NO:342: Homo sapiens Numb exon 9 sequence targeted by antisense oligonucleotide of SEQ ID NO: 340
  source 1..14: mol_type = genomic RNA
ctaatggcactgac

SEQ ID NO: 343 - RNA, 14 nt, synthetic construct
  misc_feature 1..14: note = Description for SEQ ID NO:343: Random oligonucleotide 14 nt long
  source 1..14: mol_type = other RNA
aaaccgcgcgtacg

SEQ ID NO: 344-348 - skipped (5 entries)

SEQ ID NO: 349 - RNA, 21 nt, synthetic construct
  misc_feature 1..21: note = Description for SEQ ID NO:349: Random oligonucleotide 21 nt long
  source 1..21: mol_type = other RNA
aaccgcgcgtacgaaaccgtc

SEQ ID NO: 350 - RNA, 21 nt, Homo sapiens
  misc_feature 1..21: note = Description for SEQ ID NO:350: Antisense oligonucleotide targeting SEQ ID NO: 117 in Region 1+2+2-3 of Homo sapiens Numb exon 9 21 nt long
  source 1..21: mol_type = genomic RNA
caagcacatggaaggctgagt

SEQ ID NO: 351 - RNA, 21 nt, Homo sapiens
  misc_feature 1..21: note = Description for SEQ ID NO:351: Antisense oligonucleotide targeting SEQ ID NO: 121 in Region 1+2+2-3 of Homo sapiens Numb exon 9 21 nt long
  source 1..21: mol_type = genomic RNA
ttagcaagcacatggaaggct

SEQ ID NO: 352 - RNA, 21 nt, Homo sapiens
  misc_feature 1..21: note = Description for SEQ ID NO:352: Antisense oligonucleotide targeting SEQ ID NO: 331 in Region 1+2+2-3 of Homo sapiens Numb exon 9 21 nt long
  source 1..21: mol_type = genomic RNA
gctggcttagcaagcacatgg

SEQ ID NO: 353 - RNA, 21 nt, Homo sapiens
  misc_feature 1..21: note = Description for SEQ ID NO:353: Antisense oligonucleotide targeting SEQ ID NO: in Region 2+3 of Homo sapiens Numb exon 9 21 nt long
  source 1..21: mol_type = genomic RNA
gagcagtatgggctggcttag

SEQ ID NO: 354 - RNA, 21 nt, Homo sapiens
  misc_feature 1..21: note = Description for SEQ ID NO:354: Region of Homo sapiens Numb exon 9 targeted by SEQ ID NO:353
  source 1..21: mol_type = genomic RNA
ctaagccagcccatactgctc

SEQ ID NO: 355 - RNA, 21 nt, Homo sapiens
  misc_feature 1..21: note = Description for SEQ ID NO:355: Antisense oligonucleotide targeting a in Region 2+3 of Homo sapiens Numb exon 9 21 nt long
  source 1..21: mol_type = genomic RNA
gctagagcagtatgggctggc

SEQ ID NO: 356 - RNA, 21 nt, Homo sapiens
  misc_feature 1..21: note = Description for SEQ ID NO:356: Region of Homo sapiens Numb exon 9 targeted by SEQ ID NO:355
  source 1..21: mol_type = genomic RNA
gccagcccatactgctctagc

SEQ ID NO: 357 - RNA, 21 nt, synthetic construct
  misc_feature 1..21: note = Description for SEQ ID NO:357: Random oligonucleotide 21 nt long
  source 1..21: mol_type = other RNA
tgattcgtgcggcgcgtatat